European Patent Specification EP 3 521 306 B1, published May 31, 2023. Title: Fusion protein comprising antifreeze protein and human epidermal growth factor with increased anti-oxidant activity and skin cell proliferation effect and cosmetic composition for anti-wrinkle comprising the same as effective component. Applicant: Nexgen Biotechnologies, Inc. The sequence listing filed with the application follows.

SEQUENCE LISTING (16 sequences)

SEQ ID NO: 1 - DNA, 549 bp, Artificial Sequence
  AFPSR-EGF
atgcagcgtgcacctccaaactgtccggcaggttggcaaccgctgggcgatcgttgtatctactatgagaccaccgcaatgacctgggcactggctgaaaccaactgcatgaagctgggcggccacctggcttctatccacagccaggaagaacatagctttatccagaccctgaacgcgggcgtggtctggattggtggtagcgcgtgcctgcaggctggtgcttggacttggtccgacggtactccgatgaatttccgctcctggtgctccaccaaaccggacgacgtactggctgcctgttgcatgcagatgacggcggcggccgatcagtgttgggatgacctgccgtgcccggcgtctcacaaatctgtttgcgccatgactttcaactcagactctgagtgcccactgtctcacgacggctactgccttcacgacggagtctgcatgtacatcgaggctttggataagtacgcttgtaattgcgtcgttggttacattggagagcgctgccaataccgtgacttaaaatggtgggagttgcgc

SEQ ID NO: 2 - DNA, 549 bp, Artificial Sequence
  EGF-AFPSR
atgaactcagactctgagtgcccactgtctcacgacggctactgccttcacgacggagtctgcatgtacatcgaggctttggataagtacgcttgtaattgcgtcgttggttacattggagagcgctgccaataccgtgacttaaaatggtgggagttgcgccagcgtgcacctccaaactgtccggcaggttggcaaccgctgggcgatcgttgtatctactatgagaccaccgcaatgacctgggcactggctgaaaccaactgcatgaagctgggcggccacctggcttctatccacagccaggaagaacatagctttatccagaccctgaacgcgggcgtggtctggattggtggtagcgcgtgcctgcaggctggtgcttggacttggtccgacggtactccgatgaatttccgctcctggtgctccaccaaaccggacgacgtactggctgcctgttgcatgcagatgacggcggcggccgatcagtgttgggatgacctgccgtgcccggcgtctcacaaatctgtttgcgccatgactttc

SEQ ID NO: 3 - DNA, 357 bp, Artificial Sequence
  AFPOP-EGF
atgaaccaggcatctgtggtggcaaaccagctgatccctatcaacaccgcgctgactctggtaatgatgcgcagcgaggtcgtgaccccagttggtatcccggctgaagatattccgcgtctggtttccatgcaagttaatcgtgccgtaccgctgggcacgaccctgatgccggacatggttaaaggttacgcggctaactcagactctgagtgcccactgtctcacgacggctactgccttcacgacggagtctgcatgtacatcgaggctttggataagtacgcttgtaattgcgtcgttggttacattggagagcgctgccaataccgtgacttaaaatggtgggagttgcgc

SEQ ID NO: 4 - DNA, 357 bp, Artificial Sequence
  EGF-AFPOP
atgaactcagactctgagtgcccactgtctcacgacggctactgccttcacgacggagtctgcatgtacatcgaggctttggataagtacgcttgtaattgcgtcgttggttacattggagagcgctgccaataccgtgacttaaaatggtgggagttgcgcaaccaggcatctgtggtggcaaaccagctgatccctatcaacaccgcgctgactctggtaatgatgcgcagcgaggtcgtgaccccagttggtatcccggctgaagatattccgcgtctggtttccatgcaagttaatcgtgccgtaccgctgggcacgaccctgatgccggacatggttaaaggttacgcggct

SEQ ID NO: 5 - protein, 183 aa, Artificial Sequence
  AFPSR-EGF
MQRAPPNCPAGWQPLGDRCIYYETTAMTWALAETNCMKLGGHLASIHSQEEHSFIQTLNAGVVWIGGSACLQAGAWTWSDGTPMNFRSWCSTKPDDVLAACCMQMTAAADQCWDDLPCPASHKSVCAMTFNSDSECPLSHDGYCLHDGVCMYIEALDKYACNCVVGYIGERCQYRDLKWWELR

SEQ ID NO: 6 - protein, 183 aa, Artificial Sequence
  EGF-AFPSR
MNSDSECPLSHDGYCLHDGVCMYIEALDKYACNCVVGYIGERCQYRDLKWWELRQRAPPNCPAGWQPLGDRCIYYETTAMTWALAETNCMKLGGHLASIHSQEEHSFIQTLNAGVVWIGGSACLQAGAWTWSDGTPMNFRSWCSTKPDDVLAACCMQMTAAADQCWDDLPCPASHKSVCAMTF

SEQ ID NO: 7 - protein, 119 aa, Artificial Sequence
  AFPOP-EGF
MNQASVVANQLIPINTALTLVMMRSEVVTPVGIPAEDIPRLVSMQVNRAVPLGTTLMPDMVKGYAANSDSECPLSHDGYCLHDGVCMYIEALDKYACNCVVGYIGERCQYRDLKWWELR

SEQ ID NO: 8 - protein, 119 aa, Artificial Sequence
  EGF-AFPOP
MNSDSECPLSHDGYCLHDGVCMYIEALDKYACNCVVGYIGERCQYRDLKWWELRNQASVVANQLIPINTALTLVMMRSEVVTPVGIPAEDIPRLVSMQVNRAVPLGTTLMPDMVKGYAA

SEQ ID NO: 9 - DNA, 18 bp, Artificial Sequence
  primer
atacatatgcagcgtgca

SEQ ID NO: 10 - DNA, 18 bp, Artificial Sequence
  primer
gtgctcgaggcgcaactc

SEQ ID NO: 11 - DNA, 24 bp, Artificial Sequence
  primer
cgccatgactttcaactcagactc

SEQ ID NO: 12 - DNA, 24 bp, Artificial Sequence
  primer
gtgtctgagttgaaagtcatggcg

SEQ ID NO: 13 - DNA, 18 bp, Artificial Sequence
  primer
atacatatgaaccaggca

SEQ ID NO: 14 - DNA, 15 bp, Artificial Sequence
  primer
tgctcgaggcgcaac

SEQ ID NO: 15 - DNA, 18 bp, Artificial Sequence
  primer
tacgcggctaactcagac

SEQ ID NO: 16 - DNA, 18 bp, Artificial Sequence
  primer
gtctgagttagccgcgta